European Patent Specification EP 3 975 697 B1, published September 24, 2025. Title: DOWNY MILDEW RESISTANT SPINACH PLANT. Applicant: BEJO ZADEN B.V. The sequence listing filed with the application follows.

SEQUENCE LISTING (36 sequences)

SEQ ID NO: 1 - DNA, 101 bp, Spinacia tetrandra
agggaatactggattgttggaagcgtataaattgtcaaggmccacaacaattatatgcccacgaaaataaacgcaaaagtgataactgaatacttttctac

SEQ ID NO: 2 - DNA, 101 bp, Spinacia oleracea
agggaatactggattgttggaagcgtataaattgtcaaggmccacaacaaatatatgcccacgaaaataaacgcaaaagtgataactgaatacttttctac

SEQ ID NO: 3 - DNA, 101 bp, Spinacia tetrandra
attcaaatccaaatcaaatccagaaaaattcaaaaaaaaaatacaaaatcgacgcagaaaacttacagagaatgtcgccgacgattgacgctgaaaatgcg

SEQ ID NO: 4 - DNA, 101 bp, Spinacia oleracea
attcaaatccaaatcaaatccagaaaaattcaaaaaaaaaatacaaaatcaacgcagaaaacttacagagaatgtcgccgacgattgacgctgaaaatgcg

SEQ ID NO: 5 - DNA, 101 bp, Spinacia tetrandra
atttctaccttttttacgtaccacaattccacaaacttgtgtatttatataaacactttggtcacacatttcaactacattattgcatttcatttcaatay

SEQ ID NO: 6 - DNA, 101 bp, Spinacia oleracea
atttctaccttttttacgtaccacaattccacaaacttgtgtatttatattaacactttggtcacacatttcaactacattattgcatttcatttcaatay

SEQ ID NO: 7 - DNA, 101 bp, Spinacia tetrandra
agttttctcacctgagctctgatgatagcacttttcttgtcttgctcagccttttccacaataaacttggctctttcagcatcttgtgcagctacctgttt

SEQ ID NO: 8 - DNA, 101 bp, Spinacia oleracea
agttttctcacctgagctctgatgatagcacttttcttgtcttgctcagctttttccacaataaacttggctctttcagcatcttgtgcagctacctgttt

SEQ ID NO: 9 - DNA, 101 bp, Spinacia tetrandra
tccttgataccagagatgcggttgaagacgatagctcgatgaccaccttcaacattgtacatactrtgactgactccataagcggcaaggccaagagcacc

SEQ ID NO: 10 - DNA, 101 bp, Spinacia oleracea
tccttgataccagagatgcggttgaagacgatagctcgatgaccaccttccacattgtacatactrtgactgactccataagcggcaaggccaagagcacc

SEQ ID NO: 11 - DNA, 101 bp, Spinacia tetrandra
atgcggttgaagacgatagctcgatgaccaccttcmacattgtacatactatgactgactccataagcggcaaggccaagagcaccaagaattccaacctt

SEQ ID NO: 12 - DNA, 101 bp, Spinacia oleracea
atgcggttgaagacgatagctcgatgaccaccttcmacattgtacatactgtgactgactccataagcggcaaggccaagagcaccaagaattccaacctt

SEQ ID NO: 13 - DNA, 101 bp, Spinacia tetrandra
ccataagcggcaaggccaagagcaccaagaattccaaccttaaccarattagcagcagcgccaccgccgccaccaggcatcttgggaaccttaacgttttg

SEQ ID NO: 14 - DNA, 101 bp, Spinacia oleracea
ccataagcggcaaggccaagagcaccaagaattccaaccttaaccarattggcagcagcgccaccgccgccaccaggcatcttgggaaccttaacgttttg

SEQ ID NO: 15 - DNA, 101 bp, Spinacia tetrandra
agatttctgatttcctgtagttgggagtttgattcttccagtttcggacagagaggaaaatttctcaaattatcacaaaatgtaattaacagatgagaaag

SEQ ID NO: 16 - DNA, 101 bp, Spinacia oleracea
agatttctgatttcctgtagttgggagtttgattcttccagtttcggacacagaggaaaatttctcaaattatcacaaaatgtaattaacagatgagaaag

SEQ ID NO: 17 - DNA, 101 bp, Spinacia tetrandra
aatgtgwttgaaaccctgctacttctcgtgtctcacccatatctgattctaatttccaccatccttccaactttggcatactccaaagctcaagcttttca

SEQ ID NO: 18 - DNA, 101 bp, Spinacia oleracea
aatgtgwttgaaaccctgctacttctcgtgtctcacccatatctgattctgatttccaccatccttccaactttggcatactccaaagctcaagcttttca

SEQ ID NO: 19 - DNA, 101 bp, Spinacia tetrandra
ctcctgatgttgatgcaaccccttctgcgctgatagtactattctccatatacaccacttcaytcaaatatcgtaatgtaaggaatttcaaatgacgcagt

SEQ ID NO: 20 - DNA, 101 bp, Spinacia oleracea
ctcctgatgttgatgcaaccccttctgcgctgatagtactattctccatacacaccacttcaytcaaatatcgtaatgtaaggaatttcaaatgacgcagt

SEQ ID NO: 21 - DNA, 101 bp, Spinacia tetrandra
atgcaaccccttctgcgctgatagtactattctccatayacaccacttcactcaaatatcgtaatgtaaggaatttcaaatgacgcagttgactcatcaat

SEQ ID NO: 22 - DNA, 101 bp, Spinacia oleracea
atgcaaccccttctgcgctgatagtactattctccatayacaccacttcattcaaatatcgtaatgtaaggaatttcaaatgacgcagttgactcatcaat

SEQ ID NO: 23 - DNA, 101 bp, Spinacia tetrandra
ggcatatgygacaaactcttacagccttgtatatctaggtgccttagatttactaatttcctcaaatcgcttggcaaagtttttagaccacgacactcacg

SEQ ID NO: 24 - DNA, 100 bp, Spinacia oleracea
gcatatgygacaaactcttacagccttgtatatctaggtgccttagattaactaatttcctcaaatcgcttggcaaagtttttagaccacgacactcacg

SEQ ID NO: 25 - DNA, 101 bp, Spinacia tetrandra
gatatcttagatgcaacaagttacctatctcactcggcaacatttccaaatcagagttattcaagcttaagacccttaaatattccacttttgataacaaa

SEQ ID NO: 26 - DNA, 101 bp, Spinacia oleracea
gatatcttagatgcaacaagttacctatctcactcggcaacatttccaaaccagagttattcaagcttaagacccttaaatattccacttttgataacaaa

SEQ ID NO: 27 - DNA, 101 bp, Spinacia tetrandra
tacatcatccaaaacaaggaggtatatcttcccatccagttcgtcccgaattttcatctgaagctggtccatactcatactcaggscatcgtgctttcttc

SEQ ID NO: 28 - DNA, 101 bp, Spinacia oleracea
tacatcatccaaaacaaggaggtatatcttcccatccagttcgtcccgaagtttcatctgaagctggtccatactcatactcaggscatcgtgctttcttc

SEQ ID NO: 29 - DNA, 101 bp, Spinacia tetrandra
ccagttcgtcccgaaktttcatctgaagctggtccatactcatactcagggcatcgtgctttcttctagggtttacggctgcaaggatttcagcaacaaga

SEQ ID NO: 30 - DNA, 101 bp, Spinacia oleracea
ccagttcgtcccgaaktttcatctgaagctggtccatactcatactcaggccatcgtgctttcttctagggtttacggctgcaaggatttcagcaacaaga

SEQ ID NO: 31 - DNA, 101 bp, Spinacia tetrandra
ccagccccccaatccccactatgctgacaacagaaatatccttctcctcacaagaagtgtttagtaccatatctatcactttccgcttgtcatyatccctc

SEQ ID NO: 32 - DNA, 101 bp, Spinacia oleracea
ccagccccccaatccccactatgctgacaacagaaatatccttctcctcagaagaagtgtttagtaccatatctatcactttccgcttgtcatyatccctc

SEQ ID NO: 33 - DNA, 101 bp, Spinacia tetrandra
ctcctcasaagaagtgtttagtaccatatctatcactttccgcttgtcatcatccctcccaatgatcatatcttcctcgcaaacaaaggaatgagtttccc

SEQ ID NO: 34 - DNA, 101 bp, Spinacia oleracea
ctcctcasaagaagtgtttagtaccatatctatcactttccgcttgtcattatccctcccaatgatcatatcttcctcgcaaacaaaggaatgagtttccc

SEQ ID NO: 35 - DNA, 101 bp, Spinacia tetrandra
taattgatgatttgaagatttattactacaacrcaatggattttgttttgcaattatgcattaagaagagactcrcatttttcatattggtgtatggtagt

SEQ ID NO: 36 - DNA, 101 bp, Spinacia oleracea
taattgatgatttgaagatttattactacaacrcaatggattttgttttggaattatgcattaagaagagactcrcatttttcatattggtgtatggtagt